European Patent Application EP 4 556 028 A1, published May 21, 2025. Title: Functionalized nanoparticles for viral clearance. Applicant: Leibniz-Institut für Naturstoff-Forschung und Infektionsbiologie – Hans-Knöll-Institut. Application EP. The sequence listing filed with the application follows.

SEQUENCE LISTING (2 sequences)

SEQ ID NO: 1 - protein, 30 aa, synthetic construct
MSYYHHHHHHDYDIPTTENLYFQGSGSGGS

SEQ ID NO: 2 - protein, 9 aa, synthetic construct
GSGGSGSGC